European Patent Application EP 4 726 386 A1, published April 15, 2026. Title: Methods for detecting walnut. Applicant: NISSIN FOODS HOLDINGS. Application JP PNSH-00797. The sequence listing filed with the application follows.

SEQUENCE LISTING (3 sequences)

SEQ ID NO: 1 - protein, 8 aa, Juglans regia
QSQQGQSR

SEQ ID NO: 2 - protein, 13 aa, Juglans regia
ATVVVYVVEGTGR

SEQ ID NO: 3 - protein, 8 aa, Juglans regia
ELSFNMPR